European Patent Application EP 4 737 572 A1, published May 6, 2026. Title: 去势AP205病毒样颗粒亚单位疫苗的制备方法. Applicant: 深圳赫兹生命科学技术有限公司. The sequence listing filed with the application follows.

SEQUENCE LISTING (3 sequences)

SEQ ID NO: 1 - DNA, 441 bp, synthetic construct
  source 1..441: mol_type = other DNA
atggaacactggagctacggtttgagacccggggggggcgggggatccatggcgaacaaaccgatgcaaccaattacctctacggctaataagatcgtttggtctgacccgacccgtctgtccacgacttttagcgcatctctgctgcgtcagcgcgttaaggtcggtatcgccgaactgaacaacgttagcggccagtatgtgtctgtttataaacgtccggcaccgaaaccggaaggttgtgctgatgcctgcgttatcatgccgaacgagaaccagtccatccgtaccgtgatctctggctctgcggagaacctggcaaccctgaaagctgaatgggagacccacaaacgtaatgttgataccctgtttgcctctggcaacgcaggtctgggttttctggacccaaccgctgcaattgtgtcttctgacaccaccgct

SEQ ID NO: 2 - protein, 147 aa, synthetic construct
MEHWSYGLRPGGGGGSMANKPMQPITSTANKIVWSDPTRLSTTFSASLLRQRVKVGIAELNNVSGQYVSVYKRPAPKPEGCADACVIMPNENQSIRTVISGSAENLATLKAEWETHKRNVDTLFASGNAGLGFLDPTAAIVSSDTTA

SEQ ID NO: 3 - DNA, 30 bp, synthetic construct
  source 1..30: mol_type = other DNA
atggaacactggagctacggtttgagaccc